European Patent Specification EP 3 699 264 B1, published June 7, 2023. Title: THREE-DIMENSIONAL CELL CULTURING. Applicant: UPM-KYMMENE OYJ. The sequence listing filed with the application follows.

SEQUENCE LISTING (6 sequences)

SEQ ID NO: 1 - DNA, 19 bp, Artificial Sequence
  primer
aatctccaggggcaccatt

SEQ ID NO: 2 - DNA, 18 bp, Artificial Sequence
  primer
cgctggctcccactttgt

SEQ ID NO: 3 - DNA, 20 bp, Artificial Sequence
  primer
gcagaaggcctcagcaccta

SEQ ID NO: 4 - DNA, 19 bp, Artificial Sequence
  primer
ggttcccagtcgggttcac

SEQ ID NO: 5 - DNA, 19 bp, Artificial Sequence
  primer
cagtgcccgaaacccacac

SEQ ID NO: 6 - DNA, 20 bp, Artificial Sequence
  primer
ggagacccagcagcctcaaa